European Patent Specification EP 3 619 227 B1, published August 26, 2026. Title: C-terminal CDNF and MANF fragments, pharmaceutical compositions comprising same and uses thereof. Applicant: Helsingin yliopisto. The sequence listing filed with the application follows.

SEQUENCE LISTING (10 sequences)

SEQ ID NO: 1 - protein, 81 aa, Homo sapiens [sequence omitted]

SEQ ID NO: 2 - protein, 78 aa, Homo sapiens
ICEKLKKKDSQICELKYDKQIDLSTVDLKKLRVKELKKILDDWGETCKGCAEKSDYIRKINELMPKYAPKAASARTDL

SEQ ID NO: 3 - protein, 81 aa, Homo sapiens
  VARIANT 53..54: Xaa is any amino acid
MPAMKICEKLKKLDSQICELKYEKTLDLASVDLRKMRVAELKQILHSWGEECXXCAEKTDYVNLIQELAPKYAATHPKTEL

SEQ ID NO: 4 - protein, 61 aa, Homo sapiens
KYEKTLDLASVDLRKMRVAELKQILHSWGEECRACAEKTDYVNLIQELAPKYAATHPKTEL

SEQ ID NO: 5 - protein, 63 aa, Homo sapiens
KYDKQIDLSTVDLKKLRVKELKKILDDWGETCKGCAEKSDYIRKINELMPKYAPKAASARTDL

SEQ ID NO: 6 - protein, 68 aa, Homo sapiens
  VARIANT 38..39: Xaa is any amino acid.
QICELKYDKQIDLSTVDLKKLRVKELKKILDDWGETCXXCAEKSDYIRKINELMPKYAPKAASARTDL

SEQ ID NO: 7 - protein, 161 aa, Homo sapiens
QEAGGRPGADCEVCKEFLNRFYKSLIDRGVNFSLDTIEKELISFCLDTKGKENRLCYYLGATKDAATKILSEVTRPMSVHMPAMKICEKLKKLDSQICELKYEKTLDLASVDLRKMRVAELKQILHSWGEECRACAEKTDYVNLIQELAPKYAATHPKTEL

SEQ ID NO: 8 - protein, 100 aa, Homo sapiens
QEAGGRPGADCEVCKEFLNRFYKSLIDRGVNFSLDTIEKELISFCLDTKGKENRLCYYLGATKDAATKILSEVTRPMSVHMPAMKICEKLKKLDSQICEL

SEQ ID NO: 9 - protein, 158 aa, Homo sapiens
LRPGDCEVCISYLGRFYQDLKDRDVTFSPATIENELIKFCREARGKENRLCYYIGATDDAATKIINEVSKPLAHHIPVEKICEKLKKKDSQICELKYDKQIDLSTVDLKKLRVKELKKILDDWGETCKGCAEKSDYIRKINELMPKYAPKAASARTDL

SEQ ID NO: 10 - protein, 95 aa, Homo sapiens
LRPGDCEVCISYLGRFYQDLKDRDVTFSPATIENELIKFCREARGKENRLCYYIGATDDAATKIINEVSKPLAHHIPVEKICEKLKKKDSQICEL